European Patent Application EP 4 527 929 A1, published March 26, 2025. Title: Novel Staple Nucleic Acid. Applicant: 国立大学法人　熊本大学. Application JP. The sequence listing filed with the application follows.

SEQUENCE LISTING (61 sequences)

SEQ ID NO: 1 - RNA, 373 nt, synthetic construct
  misc_feature 1..373: note = Model Target mRNA sequence "1+1 100nt RNA"
  source 1..373: mol_type = other RNA
acacaggaaacagctatgaccatgattacgccaagtttgcacgccagccgttcgacgatttaatacgactcactatagattagcatacgctactgcagtgggtaaatgtcgacctagattaatgcaattcgtgtgaagatcctttttgataatctcatgaccaaaatcccttaacgtgagttcatttccagcacccaattgaagctttaaatgggtgcatgccatgacttgcaagctattcagcaggtatacatagttggaaatctctggaagatccgcgcgtaccgagttctaattcactggccgtcgttttacaacgtcgtgactgggaaaaccctggcgttacccaacttaatcgccttgcagcacatcc

SEQ ID NO: 2 - DNA, 49 bp, synthetic construct
  misc_feature 1..49: note = (1-1) Guanine-Paying-Staple (GPS) Nucleic Acid (for 1+1 100ntRNA, type I)
  source 1..49: mol_type = other DNA
attaatctaggtcgacattttgggtgggttttaaagcttcaattgggtg

SEQ ID NO: 3 - DNA, 49 bp, synthetic construct
  misc_feature 1..49: note = (1-2) Staple_A (for 1+1 100nt RNA, type I)
  source 1..49: mol_type = other DNA
attaatctaggtcgacattttaaataaattttaaagcttcaattgggtg

SEQ ID NO: 4 - DNA, 48 bp, synthetic construct
  misc_feature 1..48: note = (1-3) Guanine-Paying-Staple (GPS) Nucleic Acid (for 1+1 100ntRNA, type II)
  source 1..48: mol_type = other DNA
gggttttacagctggatctaattagtgggttaacttcgaaattttggg

SEQ ID NO: 5 - DNA, 48 bp, synthetic construct
  misc_feature 1..48: note = (1-4) Staple_A (for 1+1 100nt RNA, type II)
  source 1..48: mol_type = other DNA
aaattttacagctggatctaattagtgggttaacttcgaaattttggg

SEQ ID NO: 6 - RNA, 373 nt, synthetic construct
  misc_feature 1..373: note = Model Target mRNA "2+1 100nt RNA"
  source 1..373: mol_type = other RNA
acacaggaaacagctatgaccatgattacgccaagtttgcacgccagccgttcgacgatttaatacgactcactatagattagcatacgctactgcagtgggtgggtgtcgacctagattaatgcaattcgtgtgaagatcctttttgataatctcatgaccaaaatcccttaacgtgagttcatttccagcacccaattgaagctttaaatgggtgcatgccatgacttgcaagctattcagcaggtatacatagttggaaatctctggaagatccgcgcgtaccgagttctaattcactggccgtcgttttacaacgtcgtgactgggaaaaccctggcgttacccaacttaatcgccttgcagcacatcc

SEQ ID NO: 7 - DNA, 45 bp, synthetic construct
  misc_feature 1..45: note = (2-1) Guanine-Paying-Staple (GPS) Nucleic Acid (for 2+1 100ntRNA)
  source 1..45: mol_type = other DNA
ttgcattaatctaggtcgactgggttttaaagcttcaattgggtg

SEQ ID NO: 8 - DNA, 45 bp, synthetic construct
  misc_feature 1..45: note = (2-2) Staple_A (for 2+1 100nt RNA)
  source 1..45: mol_type = other DNA
ttgcattaatctaggtcgactaaattttaaagcttcaattgggtg

SEQ ID NO: 9 - RNA, 373 nt, synthetic construct
  misc_feature 1..373: note = Model Target mRNA "1+1 100nt_mut 1 RNA"
  source 1..373: mol_type = other RNA
acacaggaaacagctatgaccatgattacgccaagtttgcacgccagccgttcgacgatttaatacgactcactatagattagcatacgctactgcagtgggtgaatgtcgacctagattaatgcaattcgtgtgaagatcctttttgataatctcatgaccaaaatcccttaacgtgagttcatttccagcacccaattgaagctttaagtgggtgcatgccatgacttgcaagctattcagcaggtatacatagttggaaatctctggaagatccgcgcgtaccgagttctaattcactggccgtcgttttacaacgtcgtgactgggaaaaccctggcgttacccaacttaatcgccttgcagcacatcc

SEQ ID NO: 10 - DNA, 49 bp, synthetic construct; identical to SEQ ID NO: 2
  misc_feature 1..49: note = (3-1) Guanine-Paying-Staple (GPS) Nucleic Acid (for 1+1 100nt_mut1 RNA)
  source 1..49: mol_type = other DNA

SEQ ID NO: 11 - DNA, 49 bp, synthetic construct; identical to SEQ ID NO: 3
  misc_feature 1..49: note = (3-2) Staple_A (for 1+1 100nt_mut 1 RNA)
  source 1..49: mol_type = other DNA

SEQ ID NO: 12 - RNA, 373 nt, synthetic construct
  misc_feature 1..373: note = Model Target mRNA "1+1 100nt_mut 2 RNA"
  source 1..373: mol_type = other RNA
acacaggaaacagctatgaccatgattacgccaagtttgcacgccagccgttcgacgatttaatacgactcactatagattagcatacgctactgcagtgggtggatgtcgacctagattaatgcaattcgtgtgaagatcctttttgataatctcatgaccaaaatcccttaacgtgagttcatttccagcacccaattgaagctttaagtgggtgcatgccatgacttgcaagctattcagcaggtatacatagttggaaatctctggaagatccgcgcgtaccgagttctaattcactggccgtcgttttacaacgtcgtgactgggaaaaccctggcgttacccaacttaatcgccttgcagcacatcc

SEQ ID NO: 13 - DNA, 46 bp, synthetic construct
  misc_feature 1..46: note = (4-1) Guanine-Paying-Staple (GPS) Nucleic Acid (for 1+1 100nt_mut2 RNA)
  source 1..46: mol_type = other DNA
gcattaatctaggtcgactatgtggtttaaagcttcaattgggtgc

SEQ ID NO: 14 - DNA, 46 bp, synthetic construct
  misc_feature 1..46: note = (4-2) Staple_A (for 1+1 100nt_mut 2 RNA)
  source 1..46: mol_type = other DNA
gcattaatctaggtcgactatataatttaaagcttcaattgggtgc

SEQ ID NO: 15 - RNA, 504 nt, synthetic construct
  misc_feature 1..504: note = Model Target mRNA "1+1 100nt RNA-2"
  source 1..504: mol_type = other RNA
ataccgcctcctgaaagttgtggctacaggacaggctttggctgctttctagaacgtcgctcggatccctttaaaggtggggatcttgacggagagtgcgggggatgaaggcgggagctgagggctggagagtctctgttgacatagtaactcttcagctccgtctcccttgctctccgctcttacgcttcgctaccaccagcggccccgcctgtgccctctctgcccgggcgccccagacgcatcctcgcggggtctcctcggcctgacctgctcaggtcaagatcctctttgcacccccttaagtggtgacttttccccgggccagtgggcgagccacttgcggcgggcgtctgcaccccctgcttcaccgtcgtcccctgggcaccggtctgcccaggtccagttcggccgctgacgcgaaccctccgcaccgggtccccgctggaactgcccactcggctcccccgggagcggggcccaggccagtcgggcgttcccgcc

SEQ ID NO: 16 - DNA, 49 bp, synthetic construct
  misc_feature 1..49: note = (5-1) Guanine-Paying-Staple (GPS) Nucleic Acid (for 1+1 100ntRNA-2)
  source 1..49: mol_type = other DNA
gagcaggtcaggccgaggagtgggtgggtctcccgggggagccgagtgg

SEQ ID NO: 17 - DNA, 49 bp, synthetic construct
  misc_feature 1..49: note = (5-2) Staple_A (for 1+1 100nt RNA-2)
  source 1..49: mol_type = other DNA
gagcaggtcaggccgaggagtaaataaatctcccgggggagccgagtgg

SEQ ID NO: 18 - RNA, 573 nt, Homo sapiens
  source 1..573: mol_type = mRNA
gggataccgcctcctgaaagttgtggctacaggacaggctttggctgctttctagaacgtcgctcggatccctttaaaggtggggatcttgacggagagtgcgggggatgaaggcgggagctgagggctggagagtctctgttgacatagtaactcttcagctccgtctcccttgctctccgctcttacgcttcgctaccaccagcggccccgcctgtgccctctctgcccgggcgccccagacgcatcctcgcggggtctcctcggcctgacctgctcaggtcaagatcctctttgcacccccttaagtggtgacttttccccgggccagtgggcgagccacttgcggcgggcgtctgcaccccctgcttcaccgtcgtcccctgggcaccggtctgcccaggtccagttcggccgctgacgcgaaccctccgcaccgggtccccgctggaactgcccactcggctcccccgggagcggggcccaggccagtcgggcgttcccgcccccgggtaccgagctcgaattcactggccgtcgttttacaacgtcgtgactgggaaaaccctggcg

SEQ ID NO: 19 - DNA, 51 bp, synthetic construct
  misc_feature 1..51: note = (6-1) Guanine-Paying-Staple (GPS) Nucleic Acid_T (1-1-1)
  source 1..51: mol_type = other DNA
gagcaggtcaggccgaggagtggggtggggtctcccgggggagccgagtgg

SEQ ID NO: 20 - DNA, 53 bp, synthetic construct
  misc_feature 1..53: note = (6-2) Guanine-Paying-Staple (GPS) Nucleic Acid_T (2-1-2)
  source 1..53: mol_type = other DNA
gagcaggtcaggccgaggagttggggtggggttctcccgggggagccgagtgg

SEQ ID NO: 21 - DNA, 55 bp, synthetic construct
  misc_feature 1..55: note = (6-3) Guanine-Paying-Staple (GPS) Nucleic Acid_T (3-1-3)
  source 1..55: mol_type = other DNA
gagcaggtcaggccgaggagtttggggtggggtttctcccgggggagccgagtgg

SEQ ID NO: 22 - DNA, 52 bp, synthetic construct
  misc_feature 1..52: note = (6-4) Guanine-Paying-Staple (GPS) Nucleic Acid_T (1-2-1)
  source 1..52: mol_type = other DNA
gagcaggtcaggccgaggagtggggttggggtctcccgggggagccgagtgg

SEQ ID NO: 23 - DNA, 53 bp, synthetic construct
  misc_feature 1..53: note = (6-5) Guanine-Paying-Staple (GPS) Nucleic Acid_T (1-3-1)
  source 1..53: mol_type = other DNA
gagcaggtcaggccgaggagtggggtttggggtctcccgggggagccgagtgg

SEQ ID NO: 24 - DNA, 54 bp, synthetic construct
  misc_feature 1..54: note = (6-6) Guanine-Paying-Staple (GPS) Nucleic Acid_T (2-2-2)
  source 1..54: mol_type = other DNA
gagcaggtcaggccgaggagttggggttggggttctcccgggggagccgagtgg

SEQ ID NO: 25 - DNA, 49 bp, synthetic construct
  misc_feature 1..49: note = (6-7) Guanine-Paying-Staple (GPS) Nucleic Acid_T (2-1-2)_36 mer
  source 1..49: mol_type = other DNA
gcaggtcaggccgaggagttggggtggggttctcccgggggagccgagt

SEQ ID NO: 26 - DNA, 45 bp, synthetic construct
  misc_feature 1..45: note = (6-8) Guanine-Paying-Staple (GPS) Nucleic Acid_T (2-1-2)_32 mer
  source 1..45: mol_type = other DNA
aggtcaggccgaggagttggggtggggttctcccgggggagccga

SEQ ID NO: 27 - DNA, 41 bp, synthetic construct
  misc_feature 1..41: note = (6-9) Guanine-Paying-Staple (GPS) Nucleic Acid_T (2-1-2)_28 mer
  source 1..41: mol_type = other DNA
gtcaggccgaggagttggggtggggttctcccgggggagcc

SEQ ID NO: 28 - RNA, 529 nt, Rabies
  source 1..529: mol_type = mRNA
ggctagcctcgagataccgcctcctgaaagttgtggctacaggacaggctttggctgctttctagaacgtcgctcggatccctttaaaggtggggatcttgacggagagtgcgggggatgaaggcgggagctgagggctggagagtctctgttgacatagtaactcttcagctccgtctcccttgctctccgctcttacgcttcgctaccaccagcggccccgcctgtgccctctctgcccgggcgccccagacgcatcctcgcggggtctcctcggcctgacctgctcaggtcaagatcctctttgcacccccttaagtggtgacttttccccgggccagtgggcgagccacttgcggcgggcgtctgcaccccctgcttcaccgtcgtcccctgggcaccggtctgcccaggtccagttcggccgctgacgcgaaccctccgcaccgggtccccgctggaactgcccactcggctcccccgggagcggggcccaggccagtcgggcgttcccgccgaattcgccacc

SEQ ID NO: 29 - DNA, 53 bp, synthetic construct; identical to SEQ ID NO: 20
  misc_feature 1..53: note = (7-1) Guanine-Paying-Staple (GPS) Nucleic Acid (for TRPC6 5'UTRRNA)
  source 1..53: mol_type = other DNA

SEQ ID NO: 30 - DNA, 29 bp, synthetic construct
  misc_feature 1..29: note = DNA primer for use in Stopassay on (5-1) Guanine-Paying-Staple(GPS) Nucleic Acid
  source 1..29: mol_type = other DNA
cacacaggaaacagctatgaccatgatta

SEQ ID NO: 31 - DNA, 24 bp, synthetic construct
  misc_feature 1..24: note = DNA primer for use in Stopassay on (6-1) Guanine-Paying-Staple(GPS) Nucleic Acid_T (1-1-1)
  source 1..24: mol_type = other DNA
gagatttccaactatgtatacctg

SEQ ID NO: 32 - DNA, 185 bp, synthetic construct
  misc_feature 1..185: note = PTC opti GFP
  source 1..185: mol_type = other DNA
gattagcatacgctactgcagtgggtgggtgtcgacctagattaatgcaattcgtgtgaagatcctttttgataatctcatgaccaaaatcccttaacgtgagttcatttccagcacccaattgaagctttgggtgggtgcatgccatgacttgcaagctattcagcaggtatacatagttggaa

SEQ ID NO: 33 - DNA, 30 bp, synthetic construct
  misc_feature 1..30: note = Ribosomal Shunting staple 003 (1G Staple Nucleic Acid)
  source 1..30: mol_type = other DNA
ttgtggccgtttacgttcgccggacacgct

SEQ ID NO: 34 - DNA, 720 bp, synthetic construct
  misc_feature 1..720: note = PTC GFP
  source 1..720: mol_type = other DNA
atggtgagcaagggcgaggagctgttcaccggggtggtgcccatcctggtcgtgggggacggggacgtaaacggccacaagtgaagcgtgtccggcgagggggagggggatgccacctacggcaagctgaccctgaagttcatctgcaccaccggcaagctgcccgtgccctggcccaccctcgtgaccaccctgacctacggcgtgcagtgcttcagccgctaccccgaccacatgaagcagcacgacttcttcaagtccgccatgcccgaaggctacgtccaggagcgcaccatcttcttcaaggacgacggcaactacaagacccgcgccgaggtgaagttcgagggcgacaccctggtgaaccgcatcgagctgaagggcatcgacttcaaggaggacggcaacatcctggggcacaagctggagtacaactacaacagccacaacgtctatatcatggccgacaagcagaagaacggcatcaaggtgaacttcaagatccgccacaacatcgaggacggcagcgtgcagctcgccgaccactaccagcagaacacccccatcggcgacggccccgtgctgctgcccgacaaccactacctgagcacccagtccgccctgagcaaagaccccaacgagaagcgcgatcacatggtcctgctggagttcgtgaccgccgccgggatcactctcggcatggacgagctgtacaagtaa

SEQ ID NO: 35 - DNA, 660 bp, synthetic construct
  misc_feature 1..660: note = delta type1 GFP
  source 1..660: mol_type = other DNA
atggtgagcaagggcgaggagctgttcaccggggtggtgcccatcctggtcgccacctacggcaagctgaccctgaagttcatctgcaccaccggcaagctgcccgtgccctggcccaccctcgtgaccaccctgacctacggcgtgcagtgcttcagccgctaccccgaccacatgaagcagcacgacttcttcaagtccgccatgcccgaaggctacgtccaggagcgcaccatcttcttcaaggacgacggcaactacaagacccgcgccgaggtgaagttcgagggcgacaccctggtgaaccgcatcgagctgaagggcatcgacttcaaggaggacggcaacatcctggggcacaagctggagtacaactacaacagccacaacgtctatatcatggccgacaagcagaagaacggcatcaaggtgaacttcaagatccgccacaacatcgaggacggcagcgtgcagctcgccgaccactaccagcagaacacccccatcggcgacggccccgtgctgctgcccgacaaccactacctgagcacccagtccgccctgagcaaagaccccaacgagaagcgcgatcacatggtcctgctggagttcgtgaccgccgccgggatcactctcggcatggacgagctgtacaagtaa

SEQ ID NO: 36 - DNA, 27 bp, synthetic construct
  misc_feature 1..27: note = Staple Nucleic Acid 1 (1G Staple Nucleic Acid)
  source 1..27: mol_type = other DNA
ttgtggccgtttacgttcgccggacac

SEQ ID NO: 37 - DNA, 30 bp, synthetic construct; identical to SEQ ID NO: 33
  misc_feature 1..30: note = Staple Nucleic Acid 2 (1G Staple Nucleic Acid)
  source 1..30: mol_type = other DNA

SEQ ID NO: 38 - DNA, 50 bp, synthetic construct
  source 1..50: mol_type = other DNA
gagcaggtcaggccgaggagtggggggggtctcccgggggagccgagtgg

SEQ ID NO: 39 - DNA, 52 bp, synthetic construct
  source 1..52: mol_type = other DNA
gagcaggtcaggccgaggagttggggggggttctcccgggggagccgagtgg

SEQ ID NO: 40 - DNA, 54 bp, synthetic construct
  source 1..54: mol_type = other DNA
gagcaggtcaggccgaggagtttggggggggtttctcccgggggagccgagtgg

SEQ ID NO: 41 - RNA, 853 nt, synthetic construct
  source 1..853: mol_type = other RNA
gggacagctcgaattaagaatatgtttccttgtttatcagatacatcactgcttgatgaagcaaggaagatatacatgaaaattttaaaaatacatatcgctgacttcatggaatggacatcctgtataagcactgaaaaacaacaacacaataacactaaaattttaggcactcttaaatgatctgcctctaaaagcgttggatgtagcattatgcaattaggtttttccttatttgcttcattgtactacctgtgtatatagtttttaccttttatgtagcacataaactttaaaaaaaaaaaaacaaaataaaactgaggaactgacgtggagcggggtatgaagagcttgctttgatttacagcaagtagataaatatttgacttgcatgaagagaagcaattttggggaagggtttgaattgttttctttaaagatgtaatgtccctttcagagacagctgatacttcatttaaaaaaatcacaaaaatttgaacactggctaaagataattgctatttatttttacaagaagtttattctcatttgggagatctggtgatctcccaagctatctaaagtttgttagatagctgcatgtggcttttttaaaaaagcaacagaaacctatcctcactgccctccccagtctctcttaaagttggattagcatacgctactgcagtgggtgggtgtcgacctagattaatgcaattcgtgtgaagatcctttttgataatctcatgaccaaaatcccttaacgtgagttcatttccagcacccaattgaagctttgggtgggtgcatgccatgacttgcaagctattcagctctagagtcgacctgcagg

SEQ ID NO: 42 - RNA, 853 nt, synthetic construct
  source 1..853: mol_type = other RNA
gggacagctcgaattaagaatatgtttccttgtttatcagatacatcactgcttgatgaagcaaggaagatatacatgaaaattttaaaaatacatatcgctgacttcatggaatggacatcctgtataagcactgaaaaacaacaacacaataacactaaaattttaggcactcttaaatgatctgcctctaaaagcgttggatgtagcattatgcaattaggtttttccttatttgcttcattgtactacctgtgtatatagtttttaccttttatgtagcacataaactttaaaaaaaaaaaaacaaaataaaactgaggaactgacgtggagcggggtatgaagagcttgctttgatttacagcaagtagataaatatttgacttgcatgaagagaagcaattttggggaagggtttgaattgttttctttaaagatgtaatgtccctttcagagacagctgatacttcatttaaaaaaatcacaaaaatttgaacactggctaaagataattgctatttatttttacaagaagtttattctcatttgggagatctggtgatctcccaagctatctaaagtttgttagatagctgcatgtggcttttttaaaaaagcaacagaaacctatcctcactgccctccccagtctctcttaaagttggattagcatacgctactgcagtaaataaatgtcgacctagattaatgcaattcgtgtgaagatcctttttgataatctcatgaccaaaatcccttaacgtgagttcatttccagcacccaattgaagctttaaataaatgcatgccatgacttgcaagctattcagctctagagtcgacctgcagg

SEQ ID NO: 43 - DNA, 40 bp, synthetic construct
  source 1..40: mol_type = other DNA
ttgcattaatctaggtcgacaagcttcaattgggtgctgg

SEQ ID NO: 44 - DNA, 1819 bp, synthetic construct
  source 1..1819: mol_type = other DNA
atggccgatgctaagaacattaagaagggccctgctcccttctaccctctggaggatggcaccgctggcgagcagctgcacaaggccatgaagaggtatgccctggtgcctggcaccattgccttcaccgatgcccacattgaggtggacatcacctatgccgagtacttcgagatgtctgtgcgcctggccgaggccatgaagaggtacggcctgaacaccaaccaccgcatcgtggtgtgctctgagaactctctgcagttcttcatgccagtgctgggcgccctgttcatcggagtggccgtggcccctgctaacgacatttacaacgagcgcgagctgctgaacagcatgggcatttctcagcctaccgtggtgttcgtgtctaagaagggcctgcagaagatcctgaacgtgcagaagaagctgcctatcatccagaagatcatcatcatggactctaagaccgactaccagggcttccagagcatgtacacattcgtgacatctcatctgcctcctggcttcaacgagtacgacttcgtgccagagtctttcgacagggacaaaaccattgccctgatcatgaacagctctgggtctaccggcctgcctaagggcgtggccctgcctcatcgcaccgcctgtgtgcgcttctctcacgcccgcgaccctattttcggcaaccagatcatccccgacaccgctattctgagcgtggtgccattccaccacggcttcggcatgttcaccaccctgggctacctgatttgcggctttcgggtggtgctgatgtaccgcttcgaggaggagctgttcctgcgcagcctgcaagactacaaaattcagtctgccctgctggtgccaaccctgttcagcttcttcgctaagagcaccctgatcgacaagtacgacctgtctaacctgcacgagattgcctctggcggcgccccactgtctaaggaggtgggcgaagccgtggccaagcgctttcatctgccaggcatccgccagggctacggcctgaccgagacaaccagcgccattctgattaccccagagggcgacgacaagcctggcgccgtgggcaaggtggtgccattcttcgaggccaaggtggtggacctggacaccggcaagaccctgggagtgaaccagcgcggcgagctgtgtgtgcgcggccctatgattatgtccggctacgtgaataaccctgaggccacaaacgccctgatcgacaaggacggctggctgcactctggcgacattgcctactgggacgaggacgagcacttcttcatcgtggaccgcctgaagtctctgatcaagtacaagggctaccaggtggccccagccgagctggagtctatcctgctgcagcaccctaacattttcgacgccggagtggccggcctgcccgacgacgatgccggcgagctgcctgccgccgtcgtcgtgctggaacacggcaagaccatgaccgagaaggagatcgtggactatgtggccagccaggtgacaaccgccaagaagctgcgcggcggagtggtgttcgtggacgaggtgcccaagggcctgaccggcaagctggacgcccgcaagatccgcgagatcctgatcaaggctaagaaaggcggcaagatcgccgtgtaagattagcatacgctactgcagtgggtgggtgtcgacctagattaatgcaattcgtgtgaagatcctttttgataatctcatgaccaaaatcccttaacgtgagttcatttccagcacccaattgaagctttgggtgggtgcatgccatgacttgcaagctattcag

SEQ ID NO: 45 - DNA, 40 bp, synthetic construct; identical to SEQ ID NO: 43
  source 1..40: mol_type = other DNA

SEQ ID NO: 46 - DNA, 475 bp, synthetic construct
  source 1..475: mol_type = other DNA
cacagacaaggtacttgggggggagggcagggaaatttcatattttatagtggattcttaagaaatactaacacttgagtattagcaataattacaggaaaataagtgcgaccacatatatcttaacattactgaattaaaactatggcttctaagtccttatccaaactcagtcatccaaactagtttatttttttctccagttgattatcttttaatttttaattttgctaaaggtggtttttttgtgttttgttttttgtaaaccaaaactatactaagtatagtaattatatatatatatatattttttcccctccccctcttctttcctaactaattctgagcagggtaatcagtgaacaaagtgttgaaaattgttcccagaaggtaattttcatagatgtttgcattagctccatagcaaaatggaatggtacgtgacatttagggtagctgatatttttattttgtt

SEQ ID NO: 47 - DNA, 40 bp, synthetic construct
  source 1..40: mol_type = other DNA
ccactataaaatatgaaattgctcagaattagttaggaaa

SEQ ID NO: 48 - DNA, 51 bp, synthetic construct
  source 1..51: mol_type = other DNA
caacactttgttcactgattttgggtgggttaaatgtcacgtaccattcca

SEQ ID NO: 49 - RNA, 2042 nt, synthetic construct
  source 1..2042: mol_type = other RNA
gttttcccagtcacgacgttgtaaaacgacggccagtgaattcgagctcggtacccgggtaatacgactcactatagggcctttttgataatctcatgaccaaaaatggccgatgctaagaacattaagaagggccctgctcccttctaccctctggaggatggcaccgctggcgagcagctgcacaaggccatgaagaggtatgccctggtgcctggcaccattgccttcaccgatgcccacattgaggtggacatcacctatgccgagtacttcgagatgtctgtgcgcctggccgaggccatgaagaggtacggcctgaacaccaaccaccgcatcgtggtgtgctctgagaactctctgcagttcttcatgccagtgctgggcgccctgttcatcggagtggccgtggcccctgctaacgacatttacaacgagcgcgagctgctgaacagcatgggcatttctcagcctaccgtggtgttcgtgtctaagaagggcctgcagaagatcctgaacgtgcagaagaagctgcctatcatccagaagatcatcatcatggactctaagaccgactaccagggcttccagagcatgtacacattcgtgacatctcatctgcctcctggcttcaacgagtacgacttcgtgccagagtctttcgacagggacaaaaccattgccctgatcatgaacagctctgggtctaccggcctgcctaagggcgtggccctgcctcatcgcaccgcctgtgtgcgcttctctcacgcccgcgaccctattttcggcaaccagatcatccccgacaccgctattctgagcgtggtgccattccaccacggcttcggcatgttcaccaccctgggctacctgatttgcggcttattccatggacttcatttactgggtttaacttgggtgggtgtgaagatattagcatacgctactgcagtgggtgggtgtcgacctagattaatgcaattcgtacgaagttcatagcatttccagcacccaattgaagctttgggtgggtcaagctattcagcaggtatacatagttggaaatctctggaagatccgcgcgtaccgagttctaattcactggccgtcgttttacttttgccagtagggcggcgccatggacttcatttactgggtttaacttctttcgggtggtgctgatgtaccgcttcgaggaggagctgttcctgcgcagcctgcaagactacaaaattcagtctgccctgctggtgccaaccctgttcagcttcttcgctaagagcaccctgatcgacaagtacgacctgtctaacctgcacgagattgcctctggcggcgccccactgtctaaggaggtgggcgaagccgtggccaagcgctttcatctgccaggcatccgccagggctacggcctgaccgagacaaccagcgccattctgattaccccagagggcgacgacaagcctggcgccgtgggcaaggtggtgccattcttcgaggccaaggtggtggacctggacaccggcaagaccctgggagtgaaccagcgcggcgagctgtgtgtgcgcggccctatgattatgtccggctacgtgaataaccctgaggccacaaacgccctgatcgacaaggacggctggctgcactctggcgacattgcctactgggacgaggacgagcacttcttcatcgtggaccgcctgaagtctctgatcaagtacaagggctaccaggtggccccagccgagctggagtctatcctgctgcagcaccctaacattttcgacgccggagtggccggcctgcccgacgacgatgccggcgagctgcctgccgccgtcgtcgtgctggaacacggcaagaccatgaccgagaaggagatcgtggactatgtggccagccaggtgacaaccgccaagaagctgcgcggcggagtggtgttcgtggacgaggtgcccaagggcctgaccggcaagctggacgcccgcaagatccgcgagatcctgatcaaggctaagaaaggcggcaagatcgccgtgtaa

SEQ ID NO: 50 - RNA, 39 nt, synthetic construct
  source 1..39: mol_type = other RNA
agtagcgtatgctaatatcttcacactggcaaaagtaaa

SEQ ID NO: 51 - RNA, 32 nt, synthetic construct
  source 1..32: mol_type = other RNA
tatgctaatatcttcacactggcaaaagtaaa

SEQ ID NO: 52 - RNA, 2042 nt, synthetic construct
  source 1..2042: mol_type = other RNA
gttttcccagtcacgacgttgtaaaacgacggccagtgaattcgagctcggtacccgggtaatacgactcactatagggcctttttgataatctcatgaccaaaaatggccgatgctaagaacattaagaagggccctgctcccttctaccctctggaggatggcaccgctggcgagcagctgcacaaggccatgaagaggtatgccctggtgcctggcaccattgccttcaccgatgcccacattgaggtggacatcacctatgccgagtacttcgagatgtctgtgcgcctggccgaggccatgaagaggtacggcctgaacaccaaccaccgcatcgtggtgtgctctgagaactctctgcagttcttcatgccagtgctgggcgccctgttcatcggagtggccgtggcccctgctaacgacatttacaacgagcgcgagctgctgaacagcatgggcatttctcagcctaccgtggtgttcgtgtctaagaagggcctgcagaagatcctgaacgtgcagaagaagctgcctatcatccagaagatcatcatcatggactctaagaccgactaccagggcttccagagcatgtacacattcgtgacatctcatctgcctcctggcttcaacgagtacgacttcgtgccagagtctttcgacagggacaaaaccattgccctgatcatgaacagctctgggtctaccggcctgcctaagggcgtggccctgcctcatcgcaccgcctgtgtgcgcttctctcacgcccgcgaccctattttcggcaaccagatcatccccgacaccgctattctgagcgtggtgccattccaccacggcttcggcatgttcaccaccctgggctacctgatttgcggcttattccatggacttcatttactgggtttaacttaaatgggtgtgaagatattagcatacgctactgcagtgggtgggtgtcgacctagattaatgcaattcgtacgaagttcatagcatttccagcacccaattgaagctttgggtgggtcaagctattcagcaggtatacatagttggaaatctctggaagatccgcgcgtaccgagttctaattcactggccgtcgttttacttttgccagtagggcaacaccatggacttcatttactgggtttaacttctttcgggtggtgctgatgtaccgcttcgaggaggagctgttcctgcgcagcctgcaagactacaaaattcagtctgccctgctggtgccaaccctgttcagcttcttcgctaagagcaccctgatcgacaagtacgacctgtctaacctgcacgagattgcctctggcggcgccccactgtctaaggaggtgggcgaagccgtggccaagcgctttcatctgccaggcatccgccagggctacggcctgaccgagacaaccagcgccattctgattaccccagagggcgacgacaagcctggcgccgtgggcaaggtggtgccattcttcgaggccaaggtggtggacctggacaccggcaagaccctgggagtgaaccagcgcggcgagctgtgtgtgcgcggccctatgattatgtccggctacgtgaataaccctgaggccacaaacgccctgatcgacaaggacggctggctgcactctggcgacattgcctactgggacgaggacgagcacttcttcatcgtggaccgcctgaagtctctgatcaagtacaagggctaccaggtggccccagccgagctggagtctatcctgctgcagcaccctaacattttcgacgccggagtggccggcctgcccgacgacgatgccggcgagctgcctgccgccgtcgtcgtgctggaacacggcaagaccatgaccgagaaggagatcgtggactatgtggccagccaggtgacaaccgccaagaagctgcgcggcggagtggtgttcgtggacgaggtgcccaagggcctgaccggcaagctggacgcccgcaagatccgcgagatcctgatcaaggctaagaaaggcggcaagatcgccgtgtaa

SEQ ID NO: 53 - RNA, 47 nt, synthetic construct
  source 1..47: mol_type = other RNA
agtagcgtatgctaatatcttcacgggtgggtactggcaaaagtaaa

SEQ ID NO: 54 - RNA, 1033 nt, synthetic construct
  source 1..1033: mol_type = other RNA
gttttcccagtcacgacgttgtaaaacgacggccagtgaattcgagctcggtacccgggtaatacgactcactatagggcctttttgataatctcatgaccaaaaatggccgatgctaagaacattaagaagggccctgctcccttctaccctctggaggatggcaccgctggcgagcagctgcacaaggccatgaagaggtatgccctggtgcctggcaccattgccttcaccgatgcccacattgaggtggacatcacctatgccgagtacttcgagatgtctgtgcgcctggccgaggccatgaagaggtacggcctgaacaccaaccaccgcatcgtggtgtgctctgagaactctctgcagttcttcatgccagtgctgggcgccctgttcatcggagtggccgtggcccctgctaacgacatttacaacgagcgcgagctgctgaacagcatgggcatttctcagcctaccgtggtgttcgtgtctaagaagggcctgcagaagatcctgaacgtgcagaagaagctgcctatcatccagaagatcatcatcatggactctaagaccgactaccagggcttccagagcatgtacacattcgtgacatctcatctgcctcctggcttcaacgagtacgacttcgtgccagagtctttcgacagggacaaaaccattgccctgatcatgaacagctctgggtctaccggcctgcctaagggcgtggccctgcctcatcgcaccgcctgtgtgcgcttctctcacgcccgcgaccctattttcggcaaccagatcatccccgacaccgctattctgagcgtggtgccattccaccacggcttcggcatgttcaccaccctgggctacctgatttgcggcttattccatggacttcatttactgggtttaacttgggtgggtgtgaagatattagcatacgctactgcagtgggtgggtgtcgacctagattaatgcaattcgtacgaagttcatagcatttccagcacccaattgaagctttgggtgggt

SEQ ID NO: 55 - RNA, 1041 nt, synthetic construct
  source 1..1041: mol_type = other RNA
gtggcacattgtgccacgcatgccatgacttgcaagctattcagcaggtatacatagttggaaatctctggaagatccgcgcgtaccgagttctaattcactggccgtcgttttacttttgccagtagggcggcgccatggacttcatttactgggtttaacttctttcgggtggtgctgatgtaccgcttcgaggaggagctgttcctgcgcagcctgcaagactacaaaattcagtctgccctgctggtgccaaccctgttcagcttcttcgctaagagcaccctgatcgacaagtacgacctgtctaacctgcacgagattgcctctggcggcgccccactgtctaaggaggtgggcgaagccgtggccaagcgctttcatctgccaggcatccgccagggctacggcctgaccgagacaaccagcgccattctgattaccccagagggcgacgacaagcctggcgccgtgggcaaggtggtgccattcttcgaggccaaggtggtggacctggacaccggcaagaccctgggagtgaaccagcgcggcgagctgtgtgtgcgcggccctatgattatgtccggctacgtgaataaccctgaggccacaaacgccctgatcgacaaggacggctggctgcactctggcgacattgcctactgggacgaggacgagcacttcttcatcgtggaccgcctgaagtctctgatcaagtacaagggctaccaggtggccccagccgagctggagtctatcctgctgcagcaccctaacattttcgacgccggagtggccggcctgcccgacgacgatgccggcgagctgcctgccgccgtcgtcgtgctggaacacggcaagaccatgaccgagaaggagatcgtggactatgtggccagccaggtgacaaccgccaagaagctgcgcggcggagtggtgttcgtggacgaggtgcccaagggcctgaccggcaagctggacgcccgcaagatccgcgagatcctgatcaaggctaagaaaggcggcaagatcgccgtgtaa

SEQ ID NO: 56 - RNA, 39 nt, synthetic construct; identical to SEQ ID NO: 50
  source 1..39: mol_type = other RNA

SEQ ID NO: 57 - RNA, 15 nt, synthetic construct
  source 1..15: mol_type = other RNA
actggcaaaagtaaa

SEQ ID NO: 58 - RNA, 1033 nt, synthetic construct
  source 1..1033: mol_type = other RNA
gttttcccagtcacgacgttgtaaaacgacggccagtgaattcgagctcggtacccgggtaatacgactcactatagggcctttttgataatctcatgaccaaaaatggccgatgctaagaacattaagaagggccctgctcccttctaccctctggaggatggcaccgctggcgagcagctgcacaaggccatgaagaggtatgccctggtgcctggcaccattgccttcaccgatgcccacattgaggtggacatcacctatgccgagtacttcgagatgtctgtgcgcctggccgaggccatgaagaggtacggcctgaacaccaaccaccgcatcgtggtgtgctctgagaactctctgcagttcttcatgccagtgctgggcgccctgttcatcggagtggccgtggcccctgctaacgacatttacaacgagcgcgagctgctgaacagcatgggcatttctcagcctaccgtggtgttcgtgtctaagaagggcctgcagaagatcctgaacgtgcagaagaagctgcctatcatccagaagatcatcatcatggactctaagaccgactaccagggcttccagagcatgtacacattcgtgacatctcatctgcctcctggcttcaacgagtacgacttcgtgccagagtctttcgacagggacaaaaccattgccctgatcatgaacagctctgggtctaccggcctgcctaagggcgtggccctgcctcatcgcaccgcctgtgtgcgcttctctcacgcccgcgaccctattttcggcaaccagatcatccccgacaccgctattctgagcgtggtgccattccaccacggcttcggcatgttcaccaccctgggctacctgatttgcggcttattccatggacttcatttactgggtttaacttaaatgggtgtgaagatattagcatacgctactgcagtgggtgggtgtcgacctagattaatgcaattcgtacgaagttcatagcatttccagcacccaattgaagctttgggtgggt

SEQ ID NO: 59 - RNA, 1041 nt, synthetic construct
  source 1..1041: mol_type = other RNA
gtggcacattgtgccacgcatgccatgacttgcaagctattcagcaggtatacatagttggaaatctctggaagatccgcgcgtaccgagttctaattcactggccgtcgttttacttttgccagtagggcaacaccatggacttcatttactgggtttaacttctttcgggtggtgctgatgtaccgcttcgaggaggagctgttcctgcgcagcctgcaagactacaaaattcagtctgccctgctggtgccaaccctgttcagcttcttcgctaagagcaccctgatcgacaagtacgacctgtctaacctgcacgagattgcctctggcggcgccccactgtctaaggaggtgggcgaagccgtggccaagcgctttcatctgccaggcatccgccagggctacggcctgaccgagacaaccagcgccattctgattaccccagagggcgacgacaagcctggcgccgtgggcaaggtggtgccattcttcgaggccaaggtggtggacctggacaccggcaagaccctgggagtgaaccagcgcggcgagctgtgtgtgcgcggccctatgattatgtccggctacgtgaataaccctgaggccacaaacgccctgatcgacaaggacggctggctgcactctggcgacattgcctactgggacgaggacgagcacttcttcatcgtggaccgcctgaagtctctgatcaagtacaagggctaccaggtggccccagccgagctggagtctatcctgctgcagcaccctaacattttcgacgccggagtggccggcctgcccgacgacgatgccggcgagctgcctgccgccgtcgtcgtgctggaacacggcaagaccatgaccgagaaggagatcgtggactatgtggccagccaggtgacaaccgccaagaagctgcgcggcggagtggtgttcgtggacgaggtgcccaagggcctgaccggcaagctggacgcccgcaagatccgcgagatcctgatcaaggctaagaaaggcggcaagatcgccgtgtaa

SEQ ID NO: 60 - RNA, 47 nt, synthetic construct; identical to SEQ ID NO: 53
  source 1..47: mol_type = other RNA

SEQ ID NO: 61 - RNA, 19 nt, synthetic construct
  source 1..19: mol_type = other RNA
gggtactggcaaaagtaaa